European Patent Specification EP 3 990 005 B1, published August 27, 2025. Title: DRUG PRODUCT FOR ENZYME THERAPY FOR TREATMENT OF HOMOCYSTINURIA. Applicant: ORPHAN TECHNOLOGIES, LTD. THE REGENTS OF THE UNIVERSITY OF COLORADO, A BODY CORPORATE JAN P. KRAUS RANDY WANNER DOROTHEA HOHMANN. Application PCT/USXXXX/XXXXXX. The sequence listing filed with the application follows.

SEQUENCE LISTING (5 sequences)

SEQ ID NO: 1 - protein, 412 aa, Homo sapiens
PSETPQAEVGPTGSPHRSGPHSAKGSLEKGSPEDKEAKEPLWIRPDAPSRCTWQLGRPASESPHHHTAPAKSPKILPDILKKIGDTPMVRINKIGKKFGLKCELLAKCEFFNAGGSVKDRISLRMIEDAERDGTLKPGDTIIEPTSGNTGIGLALAAAVRGYRCIIVMPEKMSSEKVDVLRALGAEIVRTPTNARFDSPESHVGVAWRLKNEIPNSHILDQYRNASNPLAHYDTTADEILQQCDGKLDMLVASVGTGGTITGIARKLKEKCPGCRIIGVDPEGSILAEPEELNQTEQTTYEVEGIGYDFIPTVLDRTVVDKWFKSNDEEAFTFARMLIAQEGLLCGGSAGSTVAVAVKAAQELQEGQRCVVILPDSVRNYMTKFLSDRWMLQKGFLKEEDLTEKKPWWWHLR

SEQ ID NO: 2 - protein, 551 aa, Homo sapiens
MPSETPQAEVGPTGCPHRSGPHSAKGSLEKGSPEDKEAKEPLWIRPDAPSRCTWQLGRPASESPHHHTAPAKSPKILPDILKKIGDTPMVRINKIGKKFGLKCELLAKCEFFNAGGSVKDRISLRMIEDAERDGTLKPGDTIIEPTSGNTGIGLALAAAVRGYRCIIVMPEKMSSEKVDVLRALGAEIVRTPTNARFDSPESHVGVAWRLKNEIPNSHILDQYRNASNPLAHYDTTADEILQQCDGKLDMLVASVGTGGTITGIARKLKEKCPGCRIIGVDPEGSILAEPEELNQTEQTTYEVEGIGYDFIPTVLDRTVVDKWFKSNDEEAFTFARMLIAQEGLLCGGSAGSTVAVAVKAAQELQEGQRCVVILPDSVRNYMTKFLSDRWMLQKGFLKEEDLTEKKPWWWHLRVQELGLSAPLTVLPTITCGHTIEILREKGFDQAPVVDEAGVILGMVTLGNMLSSLLAGKVQPSDQVGKVIYKQFKQIRLTDTLGRLSHILEMDHFALVVHEQIQYHSTGKSSQRQMVFGVVTAIDLLNFVAAQERDQK

SEQ ID NO: 3 - DNA, 1656 bp, Homo sapiens
atgccgtcagaaaccccgcaggcagaagtgggtccgacgggttgcccgcaccgtagcggtccgcattctgcaaaaggcagtctggaaaaaggttccccggaagataaagaagccaaagaaccgctgtggattcgtccggacgcaccgtcacgctgtacctggcagctgggtcgtccggcaagcgaatctccgcatcaccatacggctccggcgaaaagtccgaaaattctgccggatatcctgaagaaaattggtgacaccccgatggttcgtatcaacaaaatcggcaaaaaattcggtctgaaatgcgaactgctggctaaatgtgaatttttcaatgcgggcggttccgtgaaagatcgtatctcactgcgcatgattgaagatgctgaacgcgacggcaccctgaaaccgggtgatacgattatcgaaccgacctctggcaacacgggtatcggtctggcactggcggcggcagtccgtggttatcgctgcattatcgtgatgccggaaaaaatgagctctgaaaaagttgatgtcctgcgtgctctgggcgcggaaattgttcgtaccccgacgaatgcccgcttcgacagtccggaatcccatgtgggtgttgcatggcgcctgaaaaacgaaatcccgaattcgcacattctggatcagtatcgtaacgctagcaatccgctggcgcattacgataccacggccgacgaaatcctgcagcaatgtgatggcaaactggacatgctggtcgcttctgtgggtaccggcggtaccattacgggcatcgcgcgtaaactgaaagaaaaatgcccgggctgtcgcattatcggtgtggatccggaaggcagtattctggcggaaccggaagaactgaaccagaccgaacaaaccacgtatgaagttgaaggcatcggttacgattttattccgaccgtcctggatcgcacggtggttgacaaatggttcaaaagcaatgacgaagaagcctttaccttcgcacgtatgctgatcgctcaggaaggtctgctgtgcggtggttcagcaggttcgacggtcgcagtggcagttaaagctgcgcaggaactgcaagaaggtcaacgttgtgtcgtgattctgccggattctgttcgcaactacatgaccaaatttctgagtgaccgttggatgctgcaaaaaggcttcctgaaagaagaagatctgaccgagaaaaaaccgtggtggtggcacctgcgcgtgcaggaactgggtctgtccgcaccgctgaccgttctgccgaccatcacgtgcggccatacgattgaaatcctgcgtgaaaaaggttttgatcaggccccggttgtcgacgaagcaggcgtgattctgggtatggttaccctgggtaacatgctgagttccctgctggcgggcaaagtgcaaccgagcgatcaggttggtaaagtcatctacaaacaattcaaacagattcgtctgaccgatacgctgggccgcctgtcgcacatcctggaaatggaccatttcgcgctggttgtgcacgaacagattcaataccatagcaccggcaaatcatcgcagcgccaaatggtctttggtgtcgtgacggccattgatctgctgaatttcgtggccgcacaagaacgtgaccagaaataa

SEQ ID NO: 4 - protein, 413 aa, Artificial Sequence
  Description of Artificial Sequence: Synthetic polypeptide
MPSETPQAEVGPTGCPHRSGPHSAKGSLEKGSPEDKEAKEPLWIRPDAPSRCTWQLGRPASESPHHHTAPAKSPKILPDILKKIGDTPMVRINKIGKKFGLKCELLAKCEFFNAGGSVKDRISLRMIEDAERDGTLKPGDTIIEPTSGNTGIGLALAAAVRGYRCIIVMPEKMSSEKVDVLRALGAEIVRTPTNARFDSPESHVGVAWRLKNEIPNSHILDQYRNASNPLAHYDTTADEILQQCDGKLDMLVASVGTGGTITGIARKLKEKCPGCRIIGVDPEGSILAEPEELNQTEQTTYEVEGIGYDFIPTVLDRTVVDKWFKSNDEEAFTFARMLIAQEGLLCGGSAGSTVAVAVKAAQELQEGQRCVVILPDSVRNYMTKFLSDRWMLQKGFLKEEDLTEKKPWWWHLR

SEQ ID NO: 5 - protein, 413 aa, Artificial Sequence
  Description of Artificial Sequence: Synthetic Truncated human C15S mutant CBS polypeptide
MPSETPQAEVGPTGSPHRSGPHSAKGSLEKGSPEDKEAKEPLWIRPDAPSRCTWQLGRPASESPHHHTAPAKSPKILPDILKKIGDTPMVRINKIGKKFGLKCELLAKCEFFNAGGSVKDRISLRMIEDAERDGTLKPGDTIIEPTSGNTGIGLALAAAVRGYRCIIVMPEKMSSEKVDVLRALGAEIVRTPTNARFDSPESHVGVAWRLKNEIPNSHILDQYRNASNPLAHYDTTADEILQQCDGKLDMLVASVGTGGTITGIARKLKEKCPGCRIIGVDPEGSILAEPEELNQTEQTTYEVEGIGYDFIPTVLDRTVVDKWFKSNDEEAFTFARMLIAQEGLLCGGSAGSTVAVAVKAAQELQEGQRCVVILPDSVRNYMTKFLSDRWMLQKGFLKEEDLTEKKPWWWHLR